European Patent Application EP 4 356 932 A1, published April 24, 2024. Title: Method and drug for treating neuronal ceroid lipofuscinosis. Applicant: 清华大学. Application WO PCT/CN2022/099308, filed June 17, 2022. The sequence listing filed with the application follows.

SEQUENCE LISTING (48 sequences)

SEQ ID NO: 1 - DNA, 20 bp, synthetic construct
  misc_feature 1..20: note = GAPDH Upstream Primer
  source 1..20: mol_type = other DNA
tgcaccaccaactgcttagc

SEQ ID NO: 2 - DNA, 21 bp, synthetic construct
  misc_feature 1..21: note = GAPDH Downstream Primer
  source 1..21: mol_type = other DNA
ggcatggactgtggtcatgag

SEQ ID NO: 3 - DNA, 22 bp, synthetic construct
  misc_feature 1..22: note = CLN3 Upstream Primer
  source 1..22: mol_type = other DNA
ggttgccttttctcattctgtg

SEQ ID NO: 4 - DNA, 17 bp, synthetic construct
  misc_feature 1..17: note = CLN3 Downstream Primer
  source 1..17: mol_type = other DNA
caccaggagatcacggc

SEQ ID NO: 5 - DNA, 20 bp, synthetic construct
  misc_feature 1..20: note = SOX2 Upstream Primer
  source 1..20: mol_type = other DNA
gtcatttgctgtgggtgatg

SEQ ID NO: 6 - DNA, 20 bp, synthetic construct
  misc_feature 1..20: note = SOX2 Downstream Primer
  source 1..20: mol_type = other DNA
agaaaaacgagggaaatggg

SEQ ID NO: 7 - DNA, 21 bp, synthetic construct
  misc_feature 1..21: note = PAX6 Upstream Primer
  source 1..21: mol_type = other DNA
ccagaaaggatgcctcataaa

SEQ ID NO: 8 - DNA, 18 bp, synthetic construct
  misc_feature 1..18: note = PAX6 Downstream Primer
  source 1..18: mol_type = other DNA
tctgcgcgcccctagtta

SEQ ID NO: 9 - DNA, 20 bp, synthetic construct
  misc_feature 1..20: note = NOGGIN Upstream Primer
  source 1..20: mol_type = other DNA
tcgaacacccagaccctatc

SEQ ID NO: 10 - DNA, 20 bp, synthetic construct
  misc_feature 1..20: note = NOGGIN Downstream Primer
  source 1..20: mol_type = other DNA
catgaagcctgggtcgtagt

SEQ ID NO: 11 - DNA, 20 bp, synthetic construct
  misc_feature 1..20: note = SOX1 Upstream Primer
  source 1..20: mol_type = other DNA
caatgcggggaggagaagtc

SEQ ID NO: 12 - DNA, 20 bp, synthetic construct
  misc_feature 1..20: note = SOX1 Downstream Primer
  source 1..20: mol_type = other DNA
ctctggaccaaactgtggcg

SEQ ID NO: 13 - DNA, 19 bp, synthetic construct
  misc_feature 1..19: note = OCT4 Upstream Primer
  source 1..19: mol_type = other DNA
cagtgcccgaaacccacac

SEQ ID NO: 14 - DNA, 20 bp, synthetic construct
  misc_feature 1..20: note = OCT4 Downstream Primer
  source 1..20: mol_type = other DNA
ggagacccagcagcctcaaa

SEQ ID NO: 15 - DNA, 22 bp, synthetic construct
  misc_feature 1..22: note = KEAP1 upstream primer
  source 1..22: mol_type = other DNA
ctggaggatcataccaagcagg

SEQ ID NO: 16 - DNA, 22 bp, synthetic construct
  misc_feature 1..22: note = KEAP1 Downstream Primer
  source 1..22: mol_type = other DNA
ggataccctcaatggacaccac

SEQ ID NO: 17 - DNA, 21 bp, synthetic construct
  misc_feature 1..21: note = HMOX1 upstream primer
  source 1..21: mol_type = other DNA
aagactgcgttcctgctcaac

SEQ ID NO: 18 - DNA, 21 bp, synthetic construct
  misc_feature 1..21: note = HMOX1 Downstream Primer
  source 1..21: mol_type = other DNA
aaagccctacagcaactgtcg

SEQ ID NO: 19 - DNA, 22 bp, synthetic construct
  misc_feature 1..22: note = NQO1 upstream primer
  source 1..22: mol_type = other DNA
gaagagcactgatcgtactggc

SEQ ID NO: 20 - DNA, 21 bp, synthetic construct
  misc_feature 1..21: note = NQO1 Downstream Primer
  source 1..21: mol_type = other DNA
ggatactgaaagttcgcaggg

SEQ ID NO: 21 - DNA, 21 bp, synthetic construct
  misc_feature 1..21: note = TXNRD1 upstream primer
  source 1..21: mol_type = other DNA
taggacaagccctgcaagact

SEQ ID NO: 22 - DNA, 22 bp, synthetic construct
  misc_feature 1..22: note = TXNRD1 Downstream Primer
  source 1..22: mol_type = other DNA
ccccaattcaaagagccaatgt

SEQ ID NO: 23 - DNA, 19 bp, synthetic construct
  misc_feature 1..19: note = CTGF upstream primer
  source 1..19: mol_type = other DNA
cagcatggacgttcgtctg

SEQ ID NO: 24 - DNA, 20 bp, synthetic construct
  misc_feature 1..20: note = CTGF Downstream Primer
  source 1..20: mol_type = other DNA
aaccacggtttggtccttgg

SEQ ID NO: 25 - DNA, 22 bp, synthetic construct
  misc_feature 1..22: note = ATG5 upstream primer
  source 1..22: mol_type = other DNA
aaagatgtgcttcgagatgtgt

SEQ ID NO: 26 - DNA, 23 bp, synthetic construct
  misc_feature 1..23: note = ATG5 Downstream Primer
  source 1..23: mol_type = other DNA
cactttgtcagttaccaacgtca

SEQ ID NO: 27 - DNA, 20 bp, synthetic construct
  misc_feature 1..20: note = p62 upstream primer
  source 1..20: mol_type = other DNA
tacgacttgtgtagcgtctg

SEQ ID NO: 28 - DNA, 19 bp, synthetic construct
  misc_feature 1..19: note = p62 Downstream Primer
  source 1..19: mol_type = other DNA
cgtgtttcaccttccggag

SEQ ID NO: 29 - DNA, 21 bp, synthetic construct
  misc_feature 1..21: note = mtMinArc upstream primer
  source 1..21: mol_type = other DNA
ctaaatagcccacacgttccc

SEQ ID NO: 30 - DNA, 20 bp, synthetic construct
  misc_feature 1..20: note = mtMinArc Downstream Primer
  source 1..20: mol_type = other DNA
agagctcccgtgagtggtta

SEQ ID NO: 31 - DNA, 27 bp, synthetic construct
  misc_feature 1..27: note = b2M upstream primer
  source 1..27: mol_type = other DNA
gctgggtagctctaaacaatgtattca

SEQ ID NO: 32 - DNA, 28 bp, synthetic construct
  misc_feature 1..28: note = b2M Downstream Primer
  source 1..28: mol_type = other DNA
ccatgtactaacaaatgtctaaaatggt

SEQ ID NO: 33 - DNA, 58 bp, synthetic construct
  misc_feature 1..58: note = CLN3 shRNA Sequence
  source 1..58: mol_type = other DNA
ccggcgtagtttactttgccgagtactcgagtactcggcaaagtaaactacgtttttg

SEQ ID NO: 34 - DNA, 59 bp, synthetic construct
  misc_feature 1..59: note = KEAP1 shRNA Sequence
  source 1..59: mol_type = other DNA
ccgggcgaatgatcacagcaatgaactcgagttcattgctgtgatcattcgcttttttg

SEQ ID NO: 35 - DNA, 25 bp, synthetic construct
  misc_feature 1..25: note = sgRNA-1 Upstream Primer
  source 1..25: mol_type = other DNA
caccgaacctaagtgactaaaatcg

SEQ ID NO: 36 - DNA, 25 bp, synthetic construct
  misc_feature 1..25: note = sgRNA-1 Downstream Primer
  source 1..25: mol_type = other DNA
aaaccgattttagtcacttaggttc

SEQ ID NO: 37 - DNA, 24 bp, synthetic construct
  misc_feature 1..24: note = sgRNA-2 Upstream Primer
  source 1..24: mol_type = other DNA
caccgcagtaggcgatgggagact

SEQ ID NO: 38 - DNA, 24 bp, synthetic construct
  misc_feature 1..24: note = sgRNA-2 Downstream Primer
  source 1..24: mol_type = other DNA
aaacagtctcccatcgcctactgc

SEQ ID NO: 39 - DNA, 20 bp, synthetic construct
  misc_feature 1..20: note = up_arm Upstream Primer
  source 1..20: mol_type = other DNA
tgcaactctgtctctacggc

SEQ ID NO: 40 - DNA, 20 bp, synthetic construct
  misc_feature 1..20: note = up_arm Downstream Primer
  source 1..20: mol_type = other DNA
agcaggcttctaagggtgac

SEQ ID NO: 41 - DNA, 20 bp, synthetic construct
  misc_feature 1..20: note = down_arm Upstream Primer
  source 1..20: mol_type = other DNA
tgggagctagagcgaccatt

SEQ ID NO: 42 - DNA, 20 bp, synthetic construct
  misc_feature 1..20: note = down_arm Downstream Primer
  source 1..20: mol_type = other DNA
cggtattgctgagcgtgact

SEQ ID NO: 43 - DNA, 20 bp, synthetic construct
  misc_feature 1..20: note = CLN3_WT Upstream Primer
  source 1..20: mol_type = other DNA
agctgatactgaggaggcca

SEQ ID NO: 44 - DNA, 20 bp, synthetic construct
  misc_feature 1..20: note = CLN3_WT Downstream Primer
  source 1..20: mol_type = other DNA
gggatacccagcatggacag

SEQ ID NO: 45 - DNA, 20 bp, synthetic construct
  misc_feature 1..20: note = Puro Upstream Primer
  source 1..20: mol_type = other DNA
atgaccgagtacaagcccac

SEQ ID NO: 46 - DNA, 18 bp, synthetic construct
  misc_feature 1..18: note = Puro Downstream Primer
  source 1..18: mol_type = other DNA
tcaggcaccgggcttgcg

SEQ ID NO: 47 - DNA, 20 bp, synthetic construct
  misc_feature 1..20: note = CLN3_mut Upstream Primer
  source 1..20: mol_type = other DNA
agctctgcggtctcactcta

SEQ ID NO: 48 - DNA, 21 bp, synthetic construct
  misc_feature 1..21: note = CLN3_mut Downstream Primer
  source 1..21: mol_type = other DNA
ctggctcatacctagcgagtc